European Patent Specification EP 3 554 561 B1, published June 28, 2023. Title: CD137 BINDING FIBRONECTIN TYPE III DOMAINS. Applicant: JANSSEN BIOTECH, INC. Diem, Michael Hawkins, Rebecca Jacobs, Steven Sepulveda, Manuel. Application TO BE ASSIGNED. The sequence listing filed with the application follows.

SEQUENCE LISTING (224 sequences)

SEQ ID NO: 1 - protein, 89 aa, Artificial Sequence
  Synthetic polypeptide
LPAPKNLVVSEVTEDSLRLSWTAPDAAFDSFLIQYQESEKVGEAINLTVPGSERSYDLTGLKPGTEYTVSIYGVKGGHRSNPLSAEFTT

SEQ ID NO: 2 - protein, 94 aa, Artificial Sequence
  Synthetic polypeptide
  MOD_RES (75)..(86): Any amino acid
  MISC_FEATURE (75)..(86): This region may encompass 7-12 residues
LPAPKNLVVSEVTEDSLRLSWTAPDAAFDSFLIQYQESEKVGEAINLTVPGSERSYDLTGLKPGTEYTVSIYGVXXXXXXXXXXXXPLSAEFTT

SEQ ID NO: 3 - protein, 89 aa, Artificial Sequence
  Synthetic polypeptide
  MOD_RES (22)..(27): Ala, Arg, Asn, Asp, Glu, Gln, Gly, His, Ile, Leu, Lys, Phe, Pro, Ser, Thr, Trp, Tyr or Val
  MOD_RES (28)..(28): Phe, Ile, Leu, Val or Tyr
  MOD_RES (29)..(29): Asp, Glu or Thr
  MOD_RES (75)..(79): Ala, Arg, Asn, Asp, Glu, Gln, Gly, His, Ile, Leu, Lys, Phe, Pro, Ser, Thr, Trp, Tyr or Val
  MOD_RES (81)..(82): Ala, Arg, Asn, Asp, Glu, Gln, Gly, His, Ile, Leu, Lys, Phe, Pro, Ser, Thr, Trp, Tyr or Val
LPAPKNLVVSEVTEDSLRLSWXXXXXXXXSFLIQYQESEKVGEAINLTVPGSERSYDLTGLKPGTEYTVSIYGVXXXXXSXXLSAEFTT

SEQ ID NO: 4 - protein, 89 aa, Artificial Sequence
  Synthetic polypeptide
LPAPKNLVVSRVTEDSARLSWTAPDAAFDSFLIQYQESEKVGEAIVLTVPGSERSYDLTGLKPGTEYTVSIYGVKGGHRSNPLSAIFTT

SEQ ID NO: 5 - protein, 97 aa, Artificial Sequence
  Synthetic polypeptide
  MOD_RES (22)..(30): Ala, Asp, Glu, Phe, Gly, His, Ile, Lys, Leu, Asn, Pro, Gln, Arg, Ser, Thr, Val, Trp or Tyr
  MISC_FEATURE (22)..(30): This region may encompass 6-9 residues
  MOD_RES (78)..(87): Ala, Asp, Glu, Phe, Gly, His, Ile, Lys, Leu, Asn, Pro, Gln, Arg, Ser, Thr, Val, Trp or Tyr
  MISC_FEATURE (78)..(87): This region may encompass 7-9 residues
LPAPKNLVVSRVTEDSARLSWXXXXXXXXXFDSFLIQYQESEKVGEAIVLTVPGSERSYDLTGLKPGTEYTVSIYGVXXXXXXXXXXSNPLSAIFTT

SEQ ID NO: 6 - protein, 96 aa, Artificial Sequence
  Synthetic polypeptide
  MOD_RES (75)..(86): Ala, Asp, Glu, Phe, Gly, His, Ile, Lys, Leu, Asn, Pro, Gln, Arg, Ser, Thr, Val, Trp or Tyr
  MOD_RES (75)..(86): This region may encompass 7-12 residues
LPAPKNLVVSRVTEDSARLSWTAPDAAFDSFLIQYQESEKVGEAIVLTVPGSERSYDLTGLKPGTEYTVSIYGVXXXXXXXXXXXXSNPLSAIFTT

SEQ ID NO: 7 - protein, 89 aa, Artificial Sequence
  Description of Artificial Sequence: Synthetic polypeptide
  MOD_RES (32)..(32): Ala, Cys, Asp, Glu, Phe, Gly, His, Ile, Lys, Leu, Asn, Pro, Gln, Arg, Ser, Thr, Val, Trp, Tyr or Met
  MOD_RES (34)..(34): Ala, Cys, Asp, Glu, Phe, Gly, His, Ile, Lys, Leu, Asn, Pro, Gln, Arg, Ser, Thr, Val, Trp, Tyr or Met
  MOD_RES (36)..(36): Ala, Cys, Asp, Glu, Phe, Gly, His, Ile, Lys, Leu, Asn, Pro, Gln, Arg, Ser, Thr, Val, Trp, Tyr or Met
  MOD_RES (38)..(41): Ala, Cys, Asp, Glu, Phe, Gly, His, Ile, Lys, Leu, Asn, Pro, Gln, Arg, Ser, Thr, Val, Trp, Tyr or Met
  MOD_RES (68)..(68): Ala, Cys, Asp, Glu, Phe, Gly, His, Ile, Lys, Leu, Asn, Pro, Gln, Arg, Ser, Thr, Val, Trp, Tyr or Met
  MOD_RES (70)..(70): Ala, Cys, Asp, Glu, Phe, Gly, His, Ile, Lys, Leu, Asn, Pro, Gln, Arg, Ser, Thr, Val, Trp, Tyr or Met
  MOD_RES (72)..(72): Ala, Cys, Asp, Glu, Phe, Gly, His, Ile, Lys, Leu, Asn, Pro, Gln, Arg, Ser, Thr, Val, Trp, Tyr or Met
  MOD_RES (78)..(79): Ala, Cys, Asp, Glu, Phe, Gly, His, Ile, Lys, Leu, Asn, Pro, Gln, Arg, Ser, Thr, Val, Trp, Tyr or Met
  MOD_RES (81)..(81): Ala, Cys, Asp, Glu, Phe, Gly, His, Ile, Lys, Leu, Asn, Pro, Gln, Arg, Ser, Thr, Val, Trp, Tyr or Met
LPAPKNLVVSRVTEDSARLSWTAPDAAFDSFXIXYXEXXXXGEAIVLTVPGSERSYDLTGLKPGTEYXVXIXGVKGGXXSXPLSAIFTT

SEQ ID NO: 8 - protein, 89 aa, Artificial Sequence
  Synthetic polypeptide
  MOD_RES (32)..(32): Ala, Asp, Glu, Phe, Gly, His, Ile, Lys, Leu, Asn, Pro, Gln, Arg, Ser, Thr, Val, Tyr or Trp
  MOD_RES (34)..(34): Ala, Asp, Glu, Phe, Gly, His, Ile, Lys, Leu, Asn, Pro, Gln, Arg, Ser, Thr, Val, Tyr or Trp
  MOD_RES (36)..(36): Ala, Asp, Glu, Phe, Gly, His, Ile, Lys, Leu, Asn, Pro, Gln, Arg, Ser, Thr, Val, Tyr or Trp
  MOD_RES (38)..(41): Ala, Asp, Glu, Phe, Gly, His, Ile, Lys, Leu, Asn, Pro, Gln, Arg, Ser, Thr, Val, Tyr or Trp
  MOD_RES (46)..(46): Ala, Asp, Glu, Phe, Gly, His, Ile, Lys, Leu, Asn, Pro, Gln, Arg, Ser, Thr, Val, Tyr or Trp
  MOD_RES (48)..(48): Ala, Asp, Glu, Phe, Gly, His, Ile, Lys, Leu, Asn, Pro, Gln, Arg, Ser, Thr, Val, Tyr or Trp
  MOD_RES (68)..(68): Ala, Asp, Glu, Phe, Gly, His, Ile, Lys, Leu, Asn, Pro, Gln, Arg, Ser, Thr, Val, Tyr or Trp
  MOD_RES (70)..(70): Ala, Asp, Glu, Phe, Gly, His, Ile, Lys, Leu, Asn, Pro, Gln, Arg, Ser, Thr, Val, Tyr or Trp
  MOD_RES (72)..(72): Ala, Asp, Glu, Phe, Gly, His, Ile, Lys, Leu, Asn, Pro, Gln, Arg, Ser, Thr, Val, Tyr or Trp
  MOD_RES (78)..(79): Ala, Asp, Glu, Phe, Gly, His, Ile, Lys, Leu, Asn, Pro, Gln, Arg, Ser, Thr, Val, Tyr or Trp
  MOD_RES (81)..(81): Ala, Asp, Glu, Phe, Gly, His, Ile, Lys, Leu, Asn, Pro, Gln, Arg, Ser, Thr, Val, Tyr or Trp
  MOD_RES (84)..(84): Ala, Asp, Glu, Phe, Gly, His, Ile, Lys, Leu, Asn, Pro, Gln, Arg, Ser, Thr, Val, Tyr or Trp
  MOD_RES (86)..(86): Ala, Asp, Glu, Phe, Gly, His, Ile, Lys, Leu, Asn, Pro, Gln, Arg, Ser, Thr, Val, Tyr or Trp
LPAPKNLVVSRVTEDSARLSWTAPDAAFDSFXIXYXEXXXXGEAIXLXVPGSERSYDLTGLKPGTEYXVXIXGVKGGXXSXPLXAXFTT

SEQ ID NO: 9 - DNA, 19 bp, Artificial Sequence
  Synthetic oligonucleotide
gtgacacggcggttagaac

SEQ ID NO: 10 - DNA, 20 bp, Artificial Sequence
  Synthetic oligonucleotide
gcctttgggaagcttctaag

SEQ ID NO: 11 - DNA, 30 bp, Artificial Sequence
  Synthetic oligonucleotide
cggcggttagaacgcggctacaattaatac

SEQ ID NO: 12 - DNA, 22 bp, Artificial Sequence
  Synthetic oligonucleotide
catgattacgccaagctcagaa

SEQ ID NO: 13 - DNA, 385 bp, Artificial Sequence
  Synthetic polynucleotide
  modified_base (198)..(224): a, c, t, g, unknown or other
  misc_feature (198)..(224): n is a, c, g, or t
gtgacacggcggttagaacgcggctacaattaatacataaccccatccccctgttgacaattaatcatcggctcgtataatgtgtggaattgtgagcggataacaatttcacacaggaaacaggatctaccatgctgccggcgccgaaaaacctggttgtttctgaagttaccgaagactctctgcgtctgtcttggnnnnnnnnnnnnnnnnnnnnnnnnnnnttygactctttcctgatccagtaccaggaatctgaaaaagttggtgaagcgatcaacctgaccgttccgggttctgaacgttcttacgacctgaccggtctgaaaccgggtaccgaatacaccgtttctatctacggtgttcttagaagcttcccaaaggc

SEQ ID NO: 14 - DNA, 382 bp, Artificial Sequence
  Synthetic polynucleotide
  modified_base (198)..(221): a, c, t, g, unknown or other
  misc_feature (198)..(221): n is a, c, g, or t
gtgacacggcggttagaacgcggctacaattaatacataaccccatccccctgttgacaattaatcatcggctcgtataatgtgtggaattgtgagcggataacaatttcacacaggaaacaggatctaccatgctgccggcgccgaaaaacctggttgtttctgaagttaccgaagactctctgcgtctgtcttggnnnnnnnnnnnnnnnnnnnnnnnnttygactctttcctgatccagtaccaggaatctgaaaaagttggtgaagcgatcaacctgaccgttccgggttctgaacgttcttacgacctgaccggtctgaaaccgggtaccgaatacaccgtttctatctacggtgttcttagaagcttcccaaaggc

SEQ ID NO: 15 - DNA, 379 bp, Artificial Sequence
  Synthetic polynucleotide
  modified_base (198)..(218): a, c, t, g, unknown or other
  misc_feature (198)..(218): n is a, c, g, or t
gtgacacggcggttagaacgcggctacaattaatacataaccccatccccctgttgacaattaatcatcggctcgtataatgtgtggaattgtgagcggataacaatttcacacaggaaacaggatctaccatgctgccggcgccgaaaaacctggttgtttctgaagttaccgaagactctctgcgtctgtcttggnnnnnnnnnnnnnnnnnnnnnttygactctttcctgatccagtaccaggaatctgaaaaagttggtgaagcgatcaacctgaccgttccgggttctgaacgttcttacgacctgaccggtctgaaaccgggtaccgaatacaccgtttctatctacggtgttcttagaagcttcccaaaggc

SEQ ID NO: 16 - DNA, 376 bp, Artificial Sequence
  Synthetic polynucleotide
  modified_base (198)..(215): a, c, t, g, unknown or other
  misc_feature (198)..(215): n is a, c, g, or t
gtgacacggcggttagaacgcggctacaattaatacataaccccatccccctgttgacaattaatcatcggctcgtataatgtgtggaattgtgagcggataacaatttcacacaggaaacaggatctaccatgctgccggcgccgaaaaacctggttgtttctgaagttaccgaagactctctgcgtctgtcttggnnnnnnnnnnnnnnnnnnttygactctttcctgatccagtaccaggaatctgaaaaagttggtgaagcgatcaacctgaccgttccgggttctgaacgttcttacgacctgaccggtctgaaaccgggtaccgaatacaccgtttctatctacggtgttcttagaagcttcccaaaggc

SEQ ID NO: 17 - DNA, 131 bp, Artificial Sequence
  Synthetic polynucleotide
cggcggttagaacgcggctacaattaatacataaccccatccccctgttgacaattaatcatcggctcgtataatgtgtggaattgtgagcggataacaatttcacacaggaaacaggatctaccatgctg

SEQ ID NO: 18 - DNA, 30 bp, Artificial Sequence; identical to SEQ ID NO: 11
  Synthetic oligonucleotide

SEQ ID NO: 19 - DNA, 81 bp, Artificial Sequence
  Synthetic oligonucleotide
ccaagacagacgggcagagtcttcggtaacgcgagaaacaaccaggtttttcggcgccggcagcatggtagatcctgtttc

SEQ ID NO: 20 - DNA, 26 bp, Artificial Sequence
  Synthetic oligonucleotide
ccgaagactctgcccgtctgtcttgg

SEQ ID NO: 21 - DNA, 45 bp, Artificial Sequence
  Synthetic oligonucleotide
cagtggtctcacggattcctggtactggatcaggaaagagtcgaa

SEQ ID NO: 22 - DNA, 54 bp, Artificial Sequence
  Synthetic oligonucleotide
catgcggtctcttccgaaaaagttggtgaagcgatcgtcctgaccgttccgggt

SEQ ID NO: 23 - DNA, 29 bp, Artificial Sequence
  Synthetic oligonucleotide
ggtggtgaagatcgcagacagcgggttag

SEQ ID NO: 24 - DNA, 21 bp, Artificial Sequence
  Synthetic oligonucleotide
cggcggttagaacgcggctac

SEQ ID NO: 25 - DNA, 61 bp, Artificial Sequence
  Synthetic oligonucleotide
aagatcagttgcggccgctagactagaaccgctgccaccgccggtggtgaagatcgcagac

SEQ ID NO: 26 - DNA, 485 bp, Artificial Sequence
  Synthetic polynucleotide
  modified_base (357)..(392): a, c, t, g, unknown or other
  misc_feature (357)..(392): n is a, c, g, or t
gtgacacggcggttagaacgcggctacaattaatacataaccccatccccctgttgacaattaatcatcggctcgtataatgtgtggaattgtgagcggataacaatttcacacaggaaacaggatctaccatgctgccggcgccgaaaaacctggttgtttctcgcgttaccgaagactctgcgcgtctgtcttggaccgcgccggacgcggcgttcgactctttcctgatccagtaccaggaatctgaaaaagttggtgaagcgatcgtgctgaccgttccgggttctgaacgttcttacgacctgaccggtctgaaaccgggtaccgaatacaccgtttctatctacggtgttnnnnnnnnnnnnnnnnnnnnnnnnnnnnnnnnnnnntctaacccgctgtctgcgatcttcaccaccggcggtcaccatcaccatcaccatggcagcggttctagtctagcggccgcaactgatcttggc

SEQ ID NO: 27 - DNA, 482 bp, Artificial Sequence
  Synthetic polynucleotide
  modified_base (357)..(389): a, c, t, g, unknown or other
  misc_feature (357)..(389): n is a, c, g, or t
gtgacacggcggttagaacgcggctacaattaatacataaccccatccccctgttgacaattaatcatcggctcgtataatgtgtggaattgtgagcggataacaatttcacacaggaaacaggatctaccatgctgccggcgccgaaaaacctggttgtttctcgcgttaccgaagactctgcgcgtctgtcttggaccgcgccggacgcggcgttcgactctttcctgatccagtaccaggaatctgaaaaagttggtgaagcgatcgtgctgaccgttccgggttctgaacgttcttacgacctgaccggtctgaaaccgggtaccgaatacaccgtttctatctacggtgttnnnnnnnnnnnnnnnnnnnnnnnnnnnnnnnnntctaacccgctgtctgcgatcttcaccaccggcggtcaccatcaccatcaccatggcagcggttctagtctagcggccgcaactgatcttggc

SEQ ID NO: 28 - DNA, 479 bp, Artificial Sequence
  Synthetic polynucleotide
  modified_base (357)..(386): a, c, t, g, unknown or other
  misc_feature (357)..(386): n is a, c, g, or t
gtgacacggcggttagaacgcggctacaattaatacataaccccatccccctgttgacaattaatcatcggctcgtataatgtgtggaattgtgagcggataacaatttcacacaggaaacaggatctaccatgctgccggcgccgaaaaacctggttgtttctcgcgttaccgaagactctgcgcgtctgtcttggaccgcgccggacgcggcgttcgactctttcctgatccagtaccaggaatctgaaaaagttggtgaagcgatcgtgctgaccgttccgggttctgaacgttcttacgacctgaccggtctgaaaccgggtaccgaatacaccgtttctatctacggtgttnnnnnnnnnnnnnnnnnnnnnnnnnnnnnntctaacccgctgtctgcgatcttcaccaccggcggtcaccatcaccatcaccatggcagcggttctagtctagcggccgcaactgatcttggc

SEQ ID NO: 29 - DNA, 476 bp, Artificial Sequence
  Synthetic polynucleotide
  modified_base (357)..(383): a, c, t, g, unknown or other
  misc_feature (357)..(383): n is a, c, g, or t
gtgacacggcggttagaacgcggctacaattaatacataaccccatccccctgttgacaattaatcatcggctcgtataatgtgtggaattgtgagcggataacaatttcacacaggaaacaggatctaccatgctgccggcgccgaaaaacctggttgtttctcgcgttaccgaagactctgcgcgtctgtcttggaccgcgccggacgcggcgttcgactctttcctgatccagtaccaggaatctgaaaaagttggtgaagcgatcgtgctgaccgttccgggttctgaacgttcttacgacctgaccggtctgaaaccgggtaccgaatacaccgtttctatctacggtgttnnnnnnnnnnnnnnnnnnnnnnnnnnntctaacccgctgtctgcgatcttcaccaccggcggtcaccatcaccatcaccatggcagcggttctagtctagcggccgcaactgatcttggc

SEQ ID NO: 30 - DNA, 473 bp, Artificial Sequence
  Synthetic polynucleotide
  modified_base (357)..(380): a, c, t, g, unknown or other
  misc_feature (357)..(380): n is a, c, g, or t
gtgacacggcggttagaacgcggctacaattaatacataaccccatccccctgttgacaattaatcatcggctcgtataatgtgtggaattgtgagcggataacaatttcacacaggaaacaggatctaccatgctgccggcgccgaaaaacctggttgtttctcgcgttaccgaagactctgcgcgtctgtcttggaccgcgccggacgcggcgttcgactctttcctgatccagtaccaggaatctgaaaaagttggtgaagcgatcgtgctgaccgttccgggttctgaacgttcttacgacctgaccggtctgaaaccgggtaccgaatacaccgtttctatctacggtgttnnnnnnnnnnnnnnnnnnnnnnnntctaacccgctgtctgcgatcttcaccaccggcggtcaccatcaccatcaccatggcagcggttctagtctagcggccgcaactgatcttggc

SEQ ID NO: 31 - DNA, 470 bp, Artificial Sequence
  Synthetic polynucleotide
  modified_base (357)..(377): a, c, t, g, unknown or other
  misc_feature (357)..(377): n is a, c, g, or t
gtgacacggcggttagaacgcggctacaattaatacataaccccatccccctgttgacaattaatcatcggctcgtataatgtgtggaattgtgagcggataacaatttcacacaggaaacaggatctaccatgctgccggcgccgaaaaacctggttgtttctcgcgttaccgaagactctgcgcgtctgtcttggaccgcgccggacgcggcgttcgactctttcctgatccagtaccaggaatctgaaaaagttggtgaagcgatcgtgctgaccgttccgggttctgaacgttcttacgacctgaccggtctgaaaccgggtaccgaatacaccgtttctatctacggtgttnnnnnnnnnnnnnnnnnnnnntctaacccgctgtctgcgatcttcaccaccggcggtcaccatcaccatcaccatggcagcggttctagtctagcggccgcaactgatcttggc

SEQ ID NO: 32 - protein, 88 aa, Unknown
  3rd FN3 domain of tenascin C polypeptide
DAPSQIEVKDVTDTTALITWFKPLAEIDGIELTYGIKDVPGDRTTIDLTEDENQYSIGNLKPDTEYEVSLISRRGDMSSNPAKETFTT

SEQ ID NO: 33 - protein, 89 aa, Unknown
  Fibcon polypeptide
LDAPTDLQVTNVTDTSITVSWTPPSATITGYRITYTPSNGPGEPKELTVPPSSTSVTITGLTPGVEYVVSLYALKDNQESPPLVGTQTT

SEQ ID NO: 34 - protein, 94 aa, Unknown
  10th FN3 domain of fibronectin polypeptide
VSDVPRDLEVVAATPTSLLISWDAPAVTVRYYRITYGETGGNSPVQEFTVPGSKSTATISGLKPGVDYTITVYAVTGRGDSPASSKPISINYRT

SEQ ID NO: 35 - protein, 4 aa, Artificial Sequence
  Synthetic peptide
GSGS

SEQ ID NO: 36 - protein, 8 aa, Artificial Sequence
  Synthetic peptide
GGGSGGGS

SEQ ID NO: 37 - protein, 25 aa, Artificial Sequence
  Synthetic peptide
GGGGSGGGGSGGGGSGGGGSGGGGS

SEQ ID NO: 38 - protein, 4 aa, Artificial Sequence
  Synthetic peptide
APAP

SEQ ID NO: 39 - protein, 10 aa, Artificial Sequence
  Synthetic peptide
APAPAPAPAP

SEQ ID NO: 40 - protein, 20 aa, Artificial Sequence
  Synthetic peptide
APAPAPAPAPAPAPAPAPAP

SEQ ID NO: 41 - protein, 40 aa, Artificial Sequence
  Synthetic polypeptide
APAPAPAPAPAPAPAPAPAPAPAPAPAPAPAPAPAPAPAP

SEQ ID NO: 42 - protein, 28 aa, Artificial Sequence
  Synthetic polypeptide
EAAAKEAAAKEAAAKEAAAKEAAAKAAA

SEQ ID NO: 43 - protein, 585 aa, Artificial Sequence
  Synthetic polypeptide
DAHKSEVAHRFKDLGEENFKALVLIAFAQYLQQSPFEDHVKLVNEVTEFAKTCVADESAENCDKSLHTLFGDKLCTVATLRETYGEMADCCAKQEPERNECFLQHKDDNPNLPRLVRPEVDVMCTAFHDNEETFLKKYLYEIARRHPYFYAPELLFFAKRYKAAFTECCQAADKAACLLPKLDELRDEGKASSAKQRLKCASLQKFGERAFKAWAVARLSQRFPKAEFAEVSKLVTDLTKVHTECCHGDLLECADDRADLAKYICENQDSISSKLKECCEKPLLEKSHCIAEVENDEMPADLPSLAADFVESKDVCKNYAEAKDVFLGMFLYEYARRHPDYSVVLLLRLAKTYETTLEKCCAAADPHECYAKVFDEFKPLVEEPQNLIKQNCELFEQLGEYKFQNALLVRYTKKVPQVSTPTLVEVSRNLGKVGSKCCKHPEAKRMPCAEDYLSVVLNQLCVLHEKTPVSDRVTKCCTESLVNRRPCFSALEVDETYVPKEFNAETFTFHADICTLSEKERQIKKQTALVELVKHKPKATKEQLKAVMDDFAAFVEKCCKADDKETCFAEEGKKLVAASQAALGL

SEQ ID NO: 44 - protein, 255 aa, Homo sapiens
MGNSCYNIVATLLLVLNFERTRSLQDPCSNCPAGTFCDNNRNQICSPCPPNSFSSAGGQRTCDICRQCKGVFRTRKECSSTSNAECDCTPGFHCLGAGCSMCEQDCKQGQELTKKGCKDCCFGTFNDQKRGICRPWTNCSLDGKSVLVNGTKERDVVCGPSPADLSPGASSVTPPAPAREPGHSPQIISFFLALTSTALLFLLFFLTLRFSVVKRGRKKLLYIFKQPFMRPVQTTQEEDGCSCRFPEEEEGGCEL

SEQ ID NO: 45 - protein, 92 aa, Artificial Sequence
  CD137 Binding Centyrin
LPAPKNLVVSRVTEDSARLSWDFAYFKFDSFLIQYQESEKVGEAIVLTVPGSERSYDLTGLKPGTEYTVSIYGVGRFYTVYYSNPLSAIFTT

SEQ ID NO: 46 - protein, 94 aa, Artificial Sequence
  CD137 Binding Centyrin
LPAPKNLVVSRVTEDSARLSWSPVDADFTFDSFLIQYQESEKVGEAIVLTVPGSERSYDLTGLKPGTEYTVSIYGVGRHYTVYDSNPLSAIFTT

SEQ ID NO: 47 - protein, 95 aa, Artificial Sequence
  CD137 Binding Centyrin
LPAPKNLVVSRVTEDSARLSWKWISHEPLEFDSFLIQYQESEKVGEAIVLTVPGSERSYDLTGLKPGTEYTVSIYGVGRHYTVYDSNPLSAIFTT

SEQ ID NO: 48 - protein, 92 aa, Artificial Sequence
  CD137 Binding Centyrin
LPAPKNLVVSRVTEDSARLSWAFQWHIFDSFLIQYQESEKVGEAIVLTVPGSERSYDLTGLKPGTEYTVSIYGVGQPYTVYDSNPLSAIFTT

SEQ ID NO: 49 - protein, 93 aa, Artificial Sequence
  CD137 Binding Centyrin
LPAPKNLVVSRVTEDYARLSWKYGEHIIWFDSFLIQYQESEKVGEAIVLTVPGSERSYDLTGLKPGTEYTVSIYGVKGQHDHDSNPLSAIFTT

SEQ ID NO: 50 - protein, 92 aa, Artificial Sequence
  CD137 Binding Centyrin
LPAPKNLVVSRVTEDSARLSWTLPNIHFDSFLIQYQESEKVGEAIVLTVPGSERSYDLTGLKPGTEYTVSIYGVGRHYTVYDSNPLSAIFTT

SEQ ID NO: 51 - protein, 95 aa, Artificial Sequence
  CD137 Binding Centyrin
LPAPKNLVVSRVTEDSARLSWSQHYLSPIPFDSFLIQYQESEKVGEAIVLTVPGSERSYDLTGLKPGTEYTVSIYGVGRHYTVYDSNPLSAIFTT

SEQ ID NO: 52 - protein, 93 aa, Artificial Sequence
  CD137 Binding Centyrin
LPAPKNLVVSRVTEDSARLSWHATFGDPFDSFLIQYQESEKVGEAIVLTVPGSERSYDLTGLKPGTEYTVSIYGVGRHYTVYDSNPLSAIFTT

SEQ ID NO: 53 - protein, 93 aa, Artificial Sequence
  CD137 Binding Centyrin
LPAPKNLVVSRVTEDSARLSWNTDWVHTFDSFLIQYQESEKVGEAIVLTVPGSERSYDLTGLKPGTEYTVSIYGVGRHYTVYDSNPLSAIFTT

SEQ ID NO: 54 - protein, 95 aa, Artificial Sequence
  CD137 Binding Centyrin
LPAPKNLVVSRVTEDSARLSWTNEQITKYGFDSFLIQYQESEKVGEAIVLTVPGSERSYDLTGLKPATEYTVSIYGVGRHYTVYDSNPLSAIFTT

SEQ ID NO: 55 - protein, 95 aa, Artificial Sequence
  CD137 Binding Centyrin
LPAPKNLVVSRVTEDSARLSWDGDKWANFKFDSFLIQYQESEKVGEAIVLTVPGSERSYDLTGLKPGTEYTVSIYGVGLHYIVYDSNPLSAIFTT

SEQ ID NO: 56 - protein, 94 aa, Artificial Sequence
  CD137 Binding Centyrin
LPAPKNLVVSRVTEDSARLSWVREDAYAFDSFLIQYQESEKVGEAIVLTVPGSERSYDLTGLKPGTEYTVSIYGVSSLHWVVHDSNPLSAIFTT

SEQ ID NO: 57 - protein, 95 aa, Artificial Sequence
  CD137 Binding Centyrin
LPAPKNLVVSRVTEDSARLSWTFHPTFEGFDSFLIQYQESEKVGEAIVLTVPGSERSYDLTGLKPGTEYTVSIYGVKWTVLRPWLSNPLSAIFTT

SEQ ID NO: 58 - protein, 95 aa, Artificial Sequence
  CD137 Binding Centyrin
LPAPKNLVVSRVTEDSARLSWIRKHNHVKWFDSFLIQYQESEKVGEAIVLTVPGSERSYDLTGLKPGTEYTVSIYGVGFLIDTDDSNPLSAIFTT

SEQ ID NO: 59 - protein, 93 aa, Artificial Sequence
  CD137 Binding Centyrin
LPAPKNLVVSRVTEDSARLSWAQELDHFDSFLIQYQESEKVGEAIVLTVPGSERSYDLTGLKPGTEYTVSIYGVYWTWWVRWNSNPLSAIFTT

SEQ ID NO: 60 - protein, 96 aa, Artificial Sequence
  CD137 Binding Centyrin
LPAPKNLVVSRVTEDSARLSWTFHPTFEGFDSFLIQYQESEKVGEAIVLTVPGSERSYDLTGLKPGTEYTVSIYGVKWYAGIGYPVSNPLSAIFTT

SEQ ID NO: 61 - protein, 96 aa, Artificial Sequence
  CD137 Binding Centyrin
LPAPKNLVVSRVTEDSARLSWSEHPTPFATFDSFLIQYQESEKVGEAIVLTVPGSERSYDLTGLKPGTEYTVSIYGVWWVENHFPVSNPLSAIFTT

SEQ ID NO: 62 - protein, 94 aa, Artificial Sequence
  CD137 Binding Centyrin
LPAPKNLVVSRVTEDSARLSWEESRQFFDSFLIQYQESEKVGEAIVLTVPGSERSYDLTGLKPGTEYTVSIYGVVHRAWLRWNGSNPLSAIFTT

SEQ ID NO: 63 - protein, 95 aa, Artificial Sequence
  CD137 Binding Centyrin
LPAPKNLVVSRVTEDSARLSWDDQFEDWFDSFLIQYQESEQVGEAIVLTVPGSERSYDLTGLKPGTEYTVSIYGVHTRDWTAWNASNPLSAIFTT

SEQ ID NO: 64 - protein, 97 aa, Artificial Sequence
  CD137 Binding Centyrin
LPAPKNLVVSRVTEDSARLSWAGHYRKIRNFDSFLIQYQESEKVGEAIVLTVPGSERSYDLTGLKPGTEYTVSIYGVKFPYYYATADSNPLSAIFTT

SEQ ID NO: 65 - protein, 97 aa, Artificial Sequence
  CD137 Binding Centyrin
LPAPKNLVVSRVTEDSARLSWAGHYRKIRNFDSFLIQYQESEKVGEAIVLTVPGSKRSYDLTGLKPGTEYTVSIYGVKFPYYYATADSNPLSAIFTT

SEQ ID NO: 66 - protein, 94 aa, Artificial Sequence
  CD137 Binding Centyrin
LPAPKNLVVSRVTEDSARLSWLEGANAEFDSFLIQYQESEKVGEAIVLTVPGSERSYDLTGLKPGTEYTVSIYGVHWVGPWYPVSNPLSAIFTT

SEQ ID NO: 67 - protein, 93 aa, Artificial Sequence
  CD137 Binding Centyrin
LPAPKNLVVSRVTEDSARLSWGAKTRQFDSFLIQYQESEKVGEAIVLTVPGSERSYDLTGLKPGTEYTVSIYGVWWVENHFPVSNPLSAIFTT

SEQ ID NO: 68 - protein, 93 aa, Artificial Sequence
  CD137 Binding Centyrin
LPAPKNLVVSRVTEDSARLSWNVTQKEFDSFLIQYQESEKVGEAIVLTVPGSERSYDLTGLKPGTEYTVSIYGVGNRYYTVYDSNPLSAIFTT

SEQ ID NO: 69 - protein, 96 aa, Artificial Sequence
  CD137 Binding Centyrin
LPAPKNLVVSRVTEDSARLSWKNHTQEWEFDSFLIQYQESEKVGEAIVLTVPGSERSYDLTGLKPGTEYTVSIYGVPIAWLAWTSTSNPLSAIFTT

SEQ ID NO: 70 - protein, 97 aa, Artificial Sequence
  CD137 Binding Centyrin
LPAPKNLVVSRVTEDSARLSWNGGEYWVPRFDSFLIQYQESEKVGEAIVLTVPGSERSYDLTGLKPGTEYTVSIYGVVWLQWISWTDSNPLSAIFTT

SEQ ID NO: 71 - protein, 95 aa, Artificial Sequence
  CD137 Binding Centyrin
LPAPKNLVVSRVTEDSARLSWAVEFNPTKFDSFLIQYQESEKVGEAIVLTVPGSERSYDLTGLKPGTEYTVSIYGVWWFEQWYPVSNPLSAIFTT

SEQ ID NO: 72 - protein, 94 aa, Artificial Sequence
  CD137 Binding Centyrin
LPAPKNLVVSRVTEDSARLSWAWNRHDFDSFLIQYQESEKVGEAIVLTVPGSERSYDLTGLKPGTEYTVSIYGVHWTVLRPFIDSNPLSAIFTT

SEQ ID NO: 73 - protein, 93 aa, Artificial Sequence
  CD137 Binding Centyrin
LPAPKNLVVSRVTEDSARLSWTINSHIFDSFLIQYQESEKVGEAIVLTVPGSERSYDLTGLKPGTEYTVSIYGVWGTKYWQAQSNPLSAIFTT

SEQ ID NO: 74 - protein, 96 aa, Artificial Sequence
  CD137 Binding Centyrin
LPAPKNLVVSRVTEDSARLSWTEEDITHLRFDSFLIQYQESEKVGEAIVLTVPGSERSYDLTGLKPGTEYTVSIYGVYWTWWVRWNSNPLSAIFTT

SEQ ID NO: 75 - protein, 95 aa, Artificial Sequence
  CD137 Binding Centyrin
LPAPKNLVVSRVTEDSARLSWTKRHFYTFDSFLIQYQESEKVGEAIVLTVPGSERSYYLTGLKPGTENTVSIYGVHGNHPYTDAPANPLSAIFTT

SEQ ID NO: 76 - protein, 89 aa, Artificial Sequence
  CD137 Binding Centyrin
LPAPKNLVVSRVTEDSARLSWTAPDAAFDSFIIQYAEDSSWGEAINLHVPGSERSYDLTGLKPGTEYHVHIYGVKGGEASNPLWAWFTT

SEQ ID NO: 77 - protein, 89 aa, Artificial Sequence
  CD137 Binding Centyrin
LPAPKNLVVSRVTEDSARLSWTAPDAAFDSFYIRYWEFCHSGEAIELSVPGSERSYDLTGLKPGTEYFVRIVGVKGGRVSLPLGAKFTT

SEQ ID NO: 78 - protein, 89 aa, Artificial Sequence
  CD137 Binding Centyrin
LPAPKNLVVSRVTEDSARLSWTAPDAAFDSFEIDYWEVESEGEAIVLFVPGSERSYDLTGLKPGTEYHVHIVGVKGGTPSYPLWADFTT

SEQ ID NO: 79 - protein, 95 aa, Artificial Sequence
  CD137 Binding Centyrin
LPAPKNLVVSRVTEDSARLSWTNEQITKYGFDSFLIQYQESEKVGEAIVLTVPGSERSYDLTGLKPGTEYTVSIYGVGRHYTVYDSNPLSAIFTT

SEQ ID NO: 80 - protein, 89 aa, Artificial Sequence
  CD137 Binding Centyrin
LPAPKNLVVSRVTEDSARLSWTAPDAAFDSFEIDYWEVESEGEAIILFVPGSERSYDLTGLKPGTEYHVHIVGVKGGTPSYPLWADFTT

SEQ ID NO: 81 - protein, 89 aa, Artificial Sequence
  CD137 Binding Centyrin
LPAPKNLVVSRVTEDSARLSWTAPDAAFDSFEIPYIEVETIGEAIWLHVPGSERSYDLTGLKPGTEYSVGINGVKGGHTSNPLSARFTT

SEQ ID NO: 82 - protein, 89 aa, Artificial Sequence
  CD137 Binding Centyrin
LPAPKNLVVSRVTEDSARLSWTAPDGAFDSFEIPYIEVETIGEAIWLHVPGSERSYDLTGLKPGTEYSVGINGVKGGHTSNPLSARFTT

SEQ ID NO: 83 - protein, 89 aa, Artificial Sequence
  CD137 Binding Centyrin
LPAPKNLVVSRVTEDSARLSWTAPDAAFDSFGIPYWEWTTEGEAIQLIVPGSERSYDLTGLKPATEYHVHIVGVKGGSFSEPLPADFTT

SEQ ID NO: 84 - protein, 89 aa, Artificial Sequence
  CD137 Binding Centyrin
LPAPKNLVVSRVTEDSARLSWTAPDAAFDSFNIKYWEANLYGEAIVLTVPGSERSYGLTGLKPGTEYRVHIRGVKGGINSFPLVAVFTT

SEQ ID NO: 85 - protein, 89 aa, Artificial Sequence
  CD137 Binding Centyrin
LPAPKNLVVSRVTEDSARLSWTAPDAAFDSFYIAYWEYWGNGEAIGLIVPGSERSYDLTGLKPGTEYHVHIVGVKGGAGSVPLWANFTT

SEQ ID NO: 86 - protein, 88 aa, Artificial Sequence
  CD137 Binding Centyrin
LPAPKNLVVSHVTEDSARLSWTAPDAAFDSFEIYYLEGGRGEAIVLTVPGSERSYDLTVLKPGTEYLGTIYGVKCGWASNPLSAIFTT

SEQ ID NO: 87 - protein, 89 aa, Artificial Sequence
  CD137 Binding Centyrin
LPAPKNLVVSRVTEDSARLSWTAPDAAFDSFEIYYAEFGYYGEAIVLTVPGSERSYDLTGLKPGTEYTVTIYGVKGGWYSTPLSAIFTT

SEQ ID NO: 88 - protein, 89 aa, Artificial Sequence
  CD137 Binding Centyrin
LPAPKNLVVSRVTEDSARLSWTAPDAAFDSFSIYYGEYYNLGEAIVLTVPGSERSYDLTGLKPGTEYVVTIYGVKGGGYSNPLSAIFTT

SEQ ID NO: 89 - protein, 89 aa, Artificial Sequence
  CD137 Binding Centyrin
LPAPKNLVVSRVTEDSARLSWTAPDAAFDSFEIYYREYWYSGEAIVLTVPGSERSYDLTGLKPGTEYLVTIYGVKGGWYSDPLSAIFTT

SEQ ID NO: 90 - protein, 89 aa, Artificial Sequence
  CD137 Binding Centyrin
LPAPKNLVVSRVTEDSARLSWTAPDAAFDSFDILYLEPYQEGEAIVLTVPGSERSYDLTGLKPGTEYLVTIYGVKGGYYSLPLSAIFTT

SEQ ID NO: 91 - protein, 89 aa, Artificial Sequence
  CD137 Binding Centyrin
LPAPKNLVVSRVTEDSARLSWTAPDAAFDSFIIRYIEEGYYGEAIVLTVPGSERSYDLTGLKPGTEYHVGIEGVKGGYYSYPLSAIFTT

SEQ ID NO: 92 - protein, 88 aa, Artificial Sequence
  CD137 Binding Centyrin
LPAPKNLVVSRVTEDSARLSWTAPDGAFDSFEIYYLEGGRGEAIVLTVPGSERSYDLTGLKPGTEYLVTIYGIKCGWASNPLSAIFTT

SEQ ID NO: 93 - protein, 89 aa, Artificial Sequence
  CD137 Binding Centyrin
LPAPKNLVVSRVTEDSARLSWTAPDAAFDSFEIYYFELRLGGEAIVLTVPGSERSYDLTGLKPGTEYLVTIYGVKGGLDSQPLSAIFTT

SEQ ID NO: 94 - protein, 89 aa, Artificial Sequence
  CD137 Binding Centyrin
LPAPKNLVVSRVTEDSARLSWTAPDAAFDSFEIYYAEPRYYGEAIVLTVPGSERSYDLTGLKPGTEYTVTIYGVKGGYYSSPLSAIFTT

SEQ ID NO: 95 - protein, 89 aa, Artificial Sequence
  CD137 Binding Centyrin
LPAPKNLVVSRVTEDSARLSWTAPDAAFDSFDIYYLESWTRGEAIVLTVPGSERSYDLTGLKPGTEYLVTIYGVKGGSYSRPLSAIFTT

SEQ ID NO: 96 - protein, 89 aa, Artificial Sequence
  CD137 Binding Centyrin
LPAPKNLVVSRVTEDSARLSWTAPDAAFDSFQIYYLEQLGYGEAIVLTVPGSERSYDLTGLKPGTEYLVTIYGVKVCEQSYPLSAIFTT

SEQ ID NO: 97 - protein, 89 aa, Artificial Sequence
  CD137 Binding Centyrin
LPAPKNLVVSRVTEDSARLSWTAPDAAFDSFDIYYGEPGNLGEAIVLTVPGSERSYDLTGLKPGTEYLVTIYGVKGGDYSSPLSAIFTT

SEQ ID NO: 98 - protein, 89 aa, Artificial Sequence
  CD137 Binding Centyrin
LPAPKNLVVSRVTEDSARLSWTAPDAAFDSFDIYYYELRLGGEAIVLTVPGSERSYDLTGLKPGTEYLVTIYGVKGGYYSGPLSAIFTT

SEQ ID NO: 99 - protein, 89 aa, Artificial Sequence
  CD137 Binding Centyrin
LPAPKNLVVSRVTEDSARLSWTAPDAAFDSFDIYYRELDFQGEAIVLTVPGSERSYDLTGLKPGTEYLVIIYGVKGGSYSYTLSAIFTT

SEQ ID NO: 100 - protein, 89 aa, Artificial Sequence
  CD137 Binding Centyrin
LPAPKNLVVSRVTEDSARLSWTAPDAAFDSFYIYYREHWTIGEAIVLTVPGSERSYDLTGLKPGTEYLVTIYGVKGGAYSNPLSAIFTT

SEQ ID NO: 101 - protein, 89 aa, Artificial Sequence
  CD137 Binding Centyrin
LPAPKNLVVSRVTEDSARLSWTAPDAAFDSFSILYGEPPALGEAIVLTVPGSERSYDLTGLKPGTEYWVTIYGVKGGVFSHPLSAIFTT

SEQ ID NO: 102 - protein, 89 aa, Artificial Sequence
  CD137 Binding Centyrin
LPAPKNLVVSRVTEDSARLSWTAPDAAFDSFVIRYIEDTVMGEAIVLTVPGSERSYDLTGLKPGTEYHVSIEGVKGGPSSLPLSAIFTT

SEQ ID NO: 103 - protein, 89 aa, Artificial Sequence
  CD137 Binding Centyrin
LPAPKNLVVSRVTEDSARLSWTAPDAAFDSFNIMYLEDVQCGEAIVLTVPGSERSYDLTGLKPGTEYHVGINGVKGGLRSFPLSAIFTT

SEQ ID NO: 104 - protein, 89 aa, Artificial Sequence
  CD137 Binding Centyrin
LPAPKNLVVSRVTEDSARLSWTAPDAAFDSFRISYLEDVYYGEAIVLTVPGSERSYDLTGLKPGTEYHVGIHGVKGGIDSFPLSAIFTT

SEQ ID NO: 105 - protein, 89 aa, Artificial Sequence
  CD137 Binding Centyrin
LPAPKNLVVSRVTEDSARLSWTAPDAAFDSFDIYYGEHWKLGEAIVLTVQGSERSYDLTGLKPGTEYLVTIYGVKGGQWSFPLSAIFTT

SEQ ID NO: 106 - protein, 89 aa, Artificial Sequence
  CD137 Binding Centyrin
LPAPKNLVVSRVTEDSARLSWTAPDAAFDSFSIYYGEWHALGEAIVLTVPGSERSYDLTGLKPGTEYVVTIYGVKGGTYSLPLSAISTT

SEQ ID NO: 107 - protein, 89 aa, Artificial Sequence
  CD137 Binding Centyrin
LPAPKNLVVSRVTEDSARLSWTAPDAAFDSFSIYYGEWHALGEAIVLTVPGSERSYDLTGLKPGTEYVVTIYGVKGGTYSLPLSAIFTT

SEQ ID NO: 108 - protein, 89 aa, Artificial Sequence
  CD137 Binding Centyrin
LPAPKNLVVSRVTEDSARLSWTAPDAAFDSFNIGYYERIIPGEAIVLTVPGSERSYDLTGLKPGTEYSVLICGVKGGKGSIPLSAIFTT

SEQ ID NO: 109 - protein, 89 aa, Artificial Sequence
  CD137 Binding Centyrin
LPAPKNLVVSRVTEDSARLSWTAPDAAFDSFDIYYFEHPVGGEAIVLTVPGSERSYDLTGLKPGTEYLVTIYGVKGGYLSMPLSAIFTT

SEQ ID NO: 110 - protein, 89 aa, Artificial Sequence
  CD137 Binding Centyrin
LPAPKNLVVSRVTEDSARLSWTAPDAAFDSFEIYYMEDFHSGEAIVLTVPGSERSYDLTGLKPGTEYWVTIYGVEGGTGSLPLSAIFTT

SEQ ID NO: 111 - protein, 89 aa, Artificial Sequence
  CD137 Binding Centyrin
LPAPKNLVVSRVTEDSARLSWTAPDAAFDSFEIYYKELRAEGEAIVLTVPGSERSYDLTGLKPGTEYLVTIYGVKGGSVSIPLSAIFTT

SEQ ID NO: 112 - protein, 89 aa, Artificial Sequence
  CD137 Binding Centyrin
LPAPKNLVVSRVTEDSARLSWTAPDAAFDSFAIYYIEWTAYGEAIVLTVPGSERSYDLTGLKPGTEYVVRISGVKCGIVSFPLSAIFTT

SEQ ID NO: 113 - protein, 89 aa, Artificial Sequence
  CD137 Binding Centyrin
LPAPKNLVVSRVTEDSARLSWTAPDAAFDSFTIYYFENENGGEAIVLTVPGSERSYDLTGLKPGTEYLVTIYGVKGCDWSDPLSAIFTT

SEQ ID NO: 114 - protein, 89 aa, Artificial Sequence
  CD137 Binding Centyrin
LPAPKNLVVSRVTEDSARLSWTAPDAAFDSFDINYFEQPKGGEAIVLTVPGSERSYDLTGLKPGTEYLVTIYGVKGGPYSPPLSAIFTT

SEQ ID NO: 115 - protein, 89 aa, Artificial Sequence
  CD137 Binding Centyrin
LPAPKNLVVSRVTEDSARLSWTAPDAAFDSLQIYYFEWVVGGEAIVLTVPGSERSYDLTGLKLGTEYLVTIYGVKGGNFSDPLSAIFTT

SEQ ID NO: 116 - protein, 89 aa, Artificial Sequence
  CD137 Binding Centyrin
LPAPKNLVVSRVTEDSARLSWTAPDAAFDSFIIRYLEDISYGEAIVLTVPGSERSYDLTGLKPGTEYHVGIEGVKGGNVSFPLSAIFTT

SEQ ID NO: 117 - protein, 89 aa, Artificial Sequence
  CD137 Binding Centyrin
LPAPKNLVVSRVTEDSARLSWTAPDAAFDSFGIPYLEDIEVGEAIVLTVPGSERSYDLAGLKPGTEYHVGIYGVKGGEQSFPLSAIFTT

SEQ ID NO: 118 - protein, 89 aa, Artificial Sequence
  CD137 Binding Centyrin
LPAPKNLVVSRVTEDSARLSWTAPDAAFDSFIIRYLEDISYGEAIVLTVPGSERSYDLTGLKPGTEYHVGIEGVKGGNVSWPLSAIFTT

SEQ ID NO: 119 - protein, 89 aa, Artificial Sequence; identical to SEQ ID NO: 118
  CD137 Binding Centyrin

SEQ ID NO: 120 - protein, 87 aa, Artificial Sequence
  CD137 Binding Centyrin
LPAPKNLVVSRVTEDSARLSWTAPDAAFDSFIIYYPEYISNGEAIVLTVPGSERSYDLTGLKPGTEYHVTIGVKGGHSWPLSAIFTT

SEQ ID NO: 121 - protein, 88 aa, Artificial Sequence
  CD137 Binding Centyrin
LPAPKNLVVSRVTEDSARLSWTAPDAAFDSFLIHYTEQPSKGEAIVLTVPGSERSYDLTGLKPGTEYQVPIGVKGGTQSCPLSAIFTT

SEQ ID NO: 122 - protein, 89 aa, Artificial Sequence
  CD137 Binding Centyrin
LPAPKNLVVSRVTEDSARLSWTAPDAAFDSFTIYYFENENGGEAIVLTVPGSERSYDLTGLKPGTEYLVTIYGVKGGHWSRPLSAIFTT

SEQ ID NO: 123 - protein, 94 aa, Artificial Sequence
  CD137 Binding Centyrin
LPAPKNLVVSRVTEDSARLSWALSSVHAYFDSFLIQYQESEKVGEAIVLTVPGSERSYDLTGLKPGTEYTVSIYGVQYVDGFFKSNPLSAIFTT

SEQ ID NO: 124 - protein, 92 aa, Artificial Sequence
  CD137 Binding Centyrin
LPAPKNLVVSRVTEDSARLSWKFGEVAFDSFLIQYQESEKVGEAIVLTVPGSERSYDLTGLKPGTEYTVSIYGVGRHYTVYDSNPLSAIFTT

SEQ ID NO: 125 - protein, 92 aa, Artificial Sequence
  CD137 Binding Centyrin
LPAPKNLVVSRVTEDSARLSWAFQWHIFDSFLIQYQESEKVGEAIVLTVPGSERSYDLTGLKPGTEYTVSIYGVGRHYTVYDSNPLSAIFTT

SEQ ID NO: 126 - protein, 95 aa, Artificial Sequence
  CD137 Binding Centyrin
LPAPKNLVVSRVTEDSARLSWTNEQITKYGFDSFLIQYQESEKVGEAIVLTVPGSERSYDLTGLKPGTEYTVSIYGVGAPYTVYDSNPLSAIFTT

SEQ ID NO: 127 - protein, 93 aa, Artificial Sequence
  CD137 Binding Centyrin
LPAPKNLVVSRVTEDSARLSWRDLQYHTFDSFLIQYQESEKVGEAIVLTVPGSERSYDLTGLKPGTEYTVSIYGVGRHYTVYDSNPLSAIFTT

SEQ ID NO: 128 - protein, 92 aa, Artificial Sequence
  CD137 Binding Centyrin
LPAPKNLVVSRVTEDSARLSWPNHISIFDSFLIQYQESEKVGEAIVLTVPGSERSYDLTGLKPGTEYTVSIYGVGRFYTVFDSNPLSAIFTT

SEQ ID NO: 129 - protein, 92 aa, Artificial Sequence
  CD137 Binding Centyrin
LPAPKNLVVSRVTEDSARLSWKFHSPTFDSFLIQYQESEKVGEAIVLTVPGSERSYDLTGLKPGTEYTVSIYGVGRHYTVYDSNPLSAIVTT

SEQ ID NO: 130 - protein, 95 aa, Artificial Sequence
  CD137 Binding Centyrin
LPAPKNLVVSRVTEDSARLSWLEQEQFVNHFDSFLIQYQESEKVGEAIVLTVPGSERSYDLTGLKPGTEYTVSIYGVQYVDGFFKSNPLSAIFTT

SEQ ID NO: 131 - protein, 95 aa, Artificial Sequence
  CD137 Binding Centyrin
LPAPKNLVVSRVTEDSARLSWPLFASDLNIFDSFLIQYQESEKVGEAIVLTVPGSERSYDLTGLKPGTEYTVSIYGVGRHYTVYDSNPLSAIFTT

SEQ ID NO: 132 - protein, 95 aa, Artificial Sequence; identical to SEQ ID NO: 79
  CD137 Binding Centyrin

SEQ ID NO: 133 - protein, 94 aa, Artificial Sequence
  CD137 Binding Centyrin
LPAPKNLVVSRVTEDSARLSWRISDRLPLFDSFLIQYQESEKVGEAIVLTVPGSERSYDLTGLKPGTEYTVSIYGVGRHYTVYDSNPLSAIFTT

SEQ ID NO: 134 - protein, 93 aa, Artificial Sequence; identical to SEQ ID NO: 52
  CD137 Binding Centyrin

SEQ ID NO: 135 - protein, 95 aa, Artificial Sequence
  CD137 Binding Centyrin
LPAPKNLVVSRVTEDSARLSWTNEQITKYGFDSFLIQYQESEKVGEAIVLTVPGSERSYDLTGLKPGTEYTVSIYGVGRFYTVFDSNPLSAIFTT

SEQ ID NO: 136 - protein, 94 aa, Artificial Sequence; identical to SEQ ID NO: 72
  CD137 Binding Centyrin

SEQ ID NO: 137 - protein, 96 aa, Artificial Sequence
  CD137 Binding Centyrin
LPAPKNLVVSRVTEDSARLSWPDESRPVRFDSFLIQYQESEKVGEAIVLTVPGSERSYDLTGLKPGTEYTVSIYGVLRPWIYATNDSNPLSAIFTT

SEQ ID NO: 138 - protein, 94 aa, Artificial Sequence
  CD137 Binding Centyrin
LPAPKNLVVSRVTEDSARLSWGAITALFDSFLIQYQESEKVGEAIVLTVPGSERSYDLTGLKPGTEYTVSIYGVKFPYYYATADSNPLSAIFTT

SEQ ID NO: 139 - protein, 97 aa, Artificial Sequence; identical to SEQ ID NO: 64
  CD137 Binding Centyrin

SEQ ID NO: 140 - protein, 97 aa, Artificial Sequence
  CD137 Binding Centyrin
LPAPKNLVVSRVTEDSARLSWAGHYRKIRNFDSFLIQYQESEKVGEAIVLTVPGSERSYDLTGLKPGTEYTVSIYGVAEHWYYATQDSNPLSAIFTT

SEQ ID NO: 141 - protein, 93 aa, Artificial Sequence
  CD137 Binding Centyrin
LPAPKNLVVSRVTEDSARLSWAQSNQQFDSFLIQYQESEKVGEAIVLTVPGSERSYDLTGLKPGTEYTVSIYGVVWQNWVAYNSNPLSAIFTT

SEQ ID NO: 142 - protein, 95 aa, Artificial Sequence; identical to SEQ ID NO: 63
  CD137 Binding Centyrin

SEQ ID NO: 143 - protein, 96 aa, Artificial Sequence
  CD137 Binding Centyrin
LPAPKNLVVSRVTEDSARLSWKQVTVAPEFDSFLIQYQESEKVGEAIVLTVPGSERSYDLTGLKPGTEYTVSIYGVKFPYYYATADSNPLSAIFTT

SEQ ID NO: 144 - protein, 96 aa, Artificial Sequence
  CD137 Binding Centyrin
LPAPKNLVVSRVTEDSARLSWPDESRPVRFDSFLIQYQESEKVGEAIVLTVPGSERSYDLTGLKPGTEYTVSIYGVHTRDWTAWNASNPLSAIFTT

SEQ ID NO: 145 - protein, 96 aa, Artificial Sequence
  CD137 Binding Centyrin
LPAPKNLVVSRVTEDSARLSWNRLDSEWVAFDSFLIQYQESEKVGEAIVLTVPGSERSYDLTGLKPGTEYTVSIYGVVFRPWLAYNSNPLSAIFTT

SEQ ID NO: 146 - protein, 96 aa, Artificial Sequence
  CD137 Binding Centyrin
LPAPKNLVVSRVTEDSARLSWPDESRPVRFDSFLIQYQESEKVGEAIVLTVPGSERSYDLTGLKPGTEYTVSIYGVVGQWKYATADSNPLSAIFTT

SEQ ID NO: 147 - protein, 89 aa, Artificial Sequence
  CD137 Binding Centyrin
LPAPKNLVVSRVTEDSARLSWTAPDAAFDSFDIYYFEHPVGGEAIVLTVPGSERSYDLTGLKPGTEYLVTIYGVKGGHFSGPLSAIFTT

SEQ ID NO: 148 - protein, 89 aa, Artificial Sequence
  CD137 Binding Centyrin
LPAPKNLVVSRVTEDSARLSWTAPDAAFDSFAIQYQEYVAHGEAIVLTVPGSERSYDLTGLKPGTEYHVRISGVKGGGVSWPLSAIFTT

SEQ ID NO: 149 - protein, 89 aa, Artificial Sequence
  CD137 Binding Centyrin
LPAPKNLVVSRVTEDSARLSWTTPDAAFDSFDIYYFEHPVGGEAIVLTVPGSERSYDLTGLKPGTEYLVTIYGVKGGYLSKPLSAIFTT

SEQ ID NO: 150 - protein, 89 aa, Artificial Sequence
  CD137 Binding Centyrin
LPAPKNLIVSRVTEDSARLSWTAPDAAFDSFEIYYKELRAEGEAIVLTVPGSERSYDLTGLKPGTEYLVTIYGVKGGSVSIPLSAIFTT

SEQ ID NO: 151 - protein, 89 aa, Artificial Sequence
  CD137 Binding Centyrin
LPAPKNLVVSRVTEDSARLSWTAPDAAFDSLDIYYFEHPVGGEAIVLTVPGSERSYDLTGLKPGTEYLVTIYGVKGGYLSMPLSAIFTT

SEQ ID NO: 152 - protein, 89 aa, Artificial Sequence
  CD137 Binding Centyrin
LPAPKNLVVSHVTEDSARLSWTAPDAAFDSFDIYYFEHPVGGEAIVLTVPGSERSYDLTGLKPGTEYLVTIYGVKGGYLSMPLSAIFTT

SEQ ID NO: 153 - protein, 89 aa, Artificial Sequence
  CD137 Binding Centyrin
LPAPKNLVVSRVTEDSARLSWTAPDAAFDSFAIQYQEYVAHGEAIVLTVPGSERSYDLTGLKPGTEYHVRISGVKGGGVSWPLSAIVTT

SEQ ID NO: 154 - protein, 89 aa, Artificial Sequence
  CD137 Binding Centyrin
LLAPKNLVVSRVTEDSARLSWIAPDAAFDSFEIYYKELRAEGEAIVLTVPGSERSYDLTGLKPGTEYLVTIYGVKGGSVSIPLSAIFTT

SEQ ID NO: 155 - protein, 89 aa, Artificial Sequence
  CD137 Binding Centyrin
LPAPKNLVVSRVTEDSARLSWTAPDAAFDSFDIYYFEHPVGGEAIVLTVPGSERSYDLTGLKPGTEYLVTIYGVKGGIWSVPLSAIFTT

SEQ ID NO: 156 - protein, 89 aa, Artificial Sequence
  CD137 Binding Centyrin
LPAPKNLVVSRVTEDSARLSWTAPDAAFDSFDIYYFEHPVGGEAIVLTVPGSERSYDLTGLKPGTEYLVTIYGVKGGTYSLPLSAIFTT

SEQ ID NO: 157 - protein, 89 aa, Artificial Sequence
  CD137 Binding Centyrin
LPAPKNLVVSRVTEDSARLSWTAPDAAFDSFDIYYFEHPVGGEAIVLTVPGSERSYDLTGLKPGTEYLVTIYGVKGGELSKPLSAISTT

SEQ ID NO: 158 - protein, 89 aa, Artificial Sequence
  CD137 Binding Centyrin
LPAPKNLVVSRVTEDSARLSWTAPDAAFDSFDIYYFEHPVGGEAIVLTVPGSERSYDLTGLKPGTEYLVTIYGVKGGTYSPPLSAIFTT

SEQ ID NO: 159 - protein, 89 aa, Artificial Sequence
  CD137 Binding Centyrin
LPAPKNLVVSRVTEDSARLSWTAPDAAFDSFDIYYGEHWKLGEAIVLTVPGSERSYDLTGLKPGTEYLVTIYGVKGGMSSNPLSAIFTT

SEQ ID NO: 160 - protein, 89 aa, Artificial Sequence
  CD137 Binding Centyrin
LPAPKNLVVSRVTEDSARLSWTAPDAAFDSFDIYYFEHPVGGEAIVLTVPGSERSYDLTGLKPGTEYLVTIYGVKGGSVSIPLSAIFTT

SEQ ID NO: 161 - protein, 89 aa, Artificial Sequence
  CD137 Binding Centyrin
LPAPKNLVVSRVTEDSARLSWTAPDAAFDSFDIYYFEHPVGGEAIVLTVPGSERSYDLTGLKPGTEYLVTIYGVKGGFWSQPLSAIFTT

SEQ ID NO: 162 - protein, 89 aa, Artificial Sequence
  CD137 Binding Centyrin
LPAPKNLVVSRVTEDSARLSWTAPDAAFDSFAIIYQEYVKSGEAIVLTVPGSERSYDLTGLKPGTEYHVRIGGVKGGLLSLPLSAIFTT

SEQ ID NO: 163 - protein, 89 aa, Artificial Sequence
  CD137 Binding Centyrin
LPAPKNLVVSRVTEDSARLSWTAPDAAFDSFDIYYFEHPVGGEAIVLTVPGSERSYDLTGLKPGTEYLVTIYGVKGGELSKPLSAIFTT

SEQ ID NO: 164 - protein, 89 aa, Artificial Sequence
  CD137 Binding Centyrin
LPAPKNLVVSRVTEDSARLSWTAPDAAFDSFAIQYQEYVAHGEAIVLTVPGSERSYDLTGLKPGTEYHVRISGVKGGGVSWPLSAISTT

SEQ ID NO: 165 - protein, 89 aa, Artificial Sequence
  CD137 Binding Centyrin
LPAPKNLVVSRVTEDSAHLSWTAPDAAFDSFDIYYFEHPVGGEAIVLTVPGSERSYDLTGLKPGTEYLVTIYGVKGGYLSMPLSAIFTT

SEQ ID NO: 166 - protein, 89 aa, Artificial Sequence
  CD137 Binding Centyrin
LPAPKNLVVSRVTEDSARLSWTAPDAAFDSFHIYYGEHYNLGEAIVLTVPGSERSYDLTGLKPGTEYLVTIYGVKGGFWSTPLSAIFTT

SEQ ID NO: 167 - protein, 89 aa, Artificial Sequence; identical to SEQ ID NO: 109
  CD137 Binding Centyrin

SEQ ID NO: 168 - protein, 89 aa, Artificial Sequence
  CD137 Binding Centyrin
LPAPKNLVVSRVTEDSARLSWTAPDAAFDSFDIYYFEQPVGGEAIVLTVPGSERSYDLTGLKPGTEYLVTIYGVKGGYLSMPLSAIFTT

SEQ ID NO: 169 - protein, 89 aa, Artificial Sequence
  CD137 Binding Centyrin
LPAPKNLVVSRVTEDSARLSWTAPDAAFDSFDIYYFEHPVGGEAIVLTVPGSERSYDLTGLKPGTEYLVTIYGVKGGNFSFPLSAIFTT

SEQ ID NO: 170 - protein, 89 aa, Artificial Sequence; identical to SEQ ID NO: 109
  CD137 Binding Centyrin

SEQ ID NO: 171 - protein, 89 aa, Artificial Sequence
  CD137 Binding Centyrin
LPAPKNLVVSRVTEDSARLSWTAPDAAFDSFDIYYFEHPVGGEAIVLTVPGSERSYDLTGLKPGTEYLVTIYGVKGGNGSSPLSAIFTT

SEQ ID NO: 172 - protein, 89 aa, Artificial Sequence
  CD137 Binding Centyrin
LPAPKNLVVSRVTEDSARLSWTAPDAAFDSFDIYYFEHPVGGEAIVLTVPGSERSYDLTGLKPGTEYLVAIYGVKGGVFSHPLSAIFTT

SEQ ID NO: 173 - protein, 89 aa, Artificial Sequence; identical to SEQ ID NO: 104
  CD137 Binding Centyrin

SEQ ID NO: 174 - protein, 89 aa, Artificial Sequence
  CD137 Binding Centyrin
LPAPKNLVVSRVTEDSARLSWTAPDAAFDSFEIYYLEVRNRGEAIVLTVPGSERSYDLTGLKPGTEYHVGIAGVKGGFHSFPLSAIFTT

SEQ ID NO: 175 - protein, 89 aa, Artificial Sequence
  CD137 Binding Centyrin
LPAPKNLVVSRVTEDSARLSWTAPDAAFDSFAIQYWEGWEWGEAIVLTVPGSERSYDLTGLKPGTEYLVTIYGVKGGHWSRPLSAIFTT

SEQ ID NO: 176 - protein, 89 aa, Artificial Sequence
  CD137 Binding Centyrin
LPAPKNLVVSRVTEDSARLSWTAPDAAFDSFEIYYIEPIAPGEAIVLTVPGSERSYDLTGLKPGTEYWVTIYGVKGCDWSDPLSAIFTT

SEQ ID NO: 177 - protein, 89 aa, Artificial Sequence
  CD137 Binding Centyrin
LPAPKNLVVSRVTEDSARLSWTAPDAAFDSFEIYYFENENGGEAIVLTVPGSERSYDLTGLKPGTEYLVTIYGVKGCDWSDPLSAIFTT

SEQ ID NO: 178 - protein, 89 aa, Artificial Sequence
  CD137 Binding Centyrin
LPAPKNLVVSRVTEDSARLSWTAPDAAFDSFHIYYLEQYSRGEAIVLTVPGSERSYDLTGLKPGTEYLVTIYGVKGCDWSDPLSAIFTT

SEQ ID NO: 179 - protein, 89 aa, Artificial Sequence
  CD137 Binding Centyrin
LPAPKNLVVSRVTEDSARLSWTAPDAAFDSFQIYYFEWVVGGEAIVLTVPGSERSYDLTGLKPGTEYLVTIYGVKGCDWSDPLSAIFTT

SEQ ID NO: 180 - protein, 89 aa, Artificial Sequence
  CD137 Binding Centyrin
LPAPKNLVVSRVTEDSARLSWTAPDAAFDSFFIQYLEDVTNGEAIVLTVPGSERSYDLTGLKPGTEYRVPIAGVKGGRDSQPLSAIFTT

SEQ ID NO: 181 - protein, 89 aa, Artificial Sequence
  CD137 Binding Centyrin
LPAPKNLVVSRVTEDSARLSWTAPDAAFDSFYIRYIEDVDFGEAIVLTVPGSERSYDLTGLKPGTEYLVTIYGVKGCDWSDPLSAIFTT

SEQ ID NO: 182 - protein, 89 aa, Artificial Sequence
  CD137 Binding Centyrin
LPAPKNLVVSRVTEDSARLSWTAPDAAFDSFEIYYAEYFKNGEAIVLTVPGSERSYDLTGLKPGTEYLVTIYGVKGCDWSDPLSAISTT

SEQ ID NO: 183 - protein, 89 aa, Artificial Sequence; identical to SEQ ID NO: 118
  CD137 Binding Centyrin

SEQ ID NO: 184 - protein, 89 aa, Artificial Sequence
  CD137 Binding Centyrin
LPAPKNLVVSRVTEDSARLSWTTPDAAFDSFHIHYLEGEWGGEAIVLTVPGSERSYDLTGLKPGTEYLVTIYGVKGCDWSDPLSAIFTT

SEQ ID NO: 185 - protein, 89 aa, Artificial Sequence
  CD137 Binding Centyrin
LPAPKNLVVSRVTEDSARLSWTAPDAAFDSFDINYFENELGGEAIVLTVPGSERSYDLTGLKPGTEYLVTIYGVKGCDWSDPLSAIFTT

SEQ ID NO: 186 - protein, 89 aa, Artificial Sequence; identical to SEQ ID NO: 122
  CD137 Binding Centyrin

SEQ ID NO: 187 - protein, 89 aa, Artificial Sequence; identical to SEQ ID NO: 113
  CD137 Binding Centyrin

SEQ ID NO: 188 - protein, 89 aa, Artificial Sequence
  CD137 Binding Centyrin
LPAPKNLVVSRVTEDSARLSWTAPDAAFDSFTIYYFENENGGEAIVLTVPGSERSYDLTGLKPDTEYLVTIYGVKGGHWSRPLSAIFTT

SEQ ID NO: 189 - protein, 89 aa, Artificial Sequence
  CD137 Binding Centyrin
LPAPKNLVVSRVTEDSARLSWTAPDAAFDSFEIYYFENELGGEAIVLTVPGSERSYDLTGLKPGTEYLVTIYGVKGGDWSDPLSAIFTT

SEQ ID NO: 190 - protein, 89 aa, Artificial Sequence
  CD137 Binding Centyrin
LPAPKNLVVSRVTEDSARLSWTAPDAAFDSFHIHYLEGEWGGEAIVLTVPGSERSYDLTGLKPGTEYLVTIYGVKGCDWSDPLSAIFTT

SEQ ID NO: 191 - protein, 89 aa, Artificial Sequence
  CD137 Binding Centyrin
LPAPKNLVVSRVTEDSARLSWTAPDAAFDSFEIYYFENELGGEAIVLTVPGSERSYDLTGLKPGTEYLVTIYGVKGCDWSDPLSAIFTT

SEQ ID NO: 192 - protein, 89 aa, Artificial Sequence
  CD137 Binding Centyrin
LPAPKNLFVSRVTEDSARLSWTAPDAAFDSFQIYYREQWWDGEAIVLTVPGSERSYDLTGLKPGTEYLVTIYGVKGCDWSDPLSAIFTT

SEQ ID NO: 193 - protein, 89 aa, Artificial Sequence
  CD137 Binding Centyrin
LPAPKNLVVSRVTEDSARLSWTAPDAAFDSFDINYFEQPKGGEAIVLTVPGSERSYDLTGLKPGTEYLVTIYGVKGCDWSDPLSAIFTT

SEQ ID NO: 194 - protein, 89 aa, Artificial Sequence
  CD137 Binding Centyrin
LPAPKNLVVSRVTEDSARLSWTAPDAAFDSFEIYYDELRNPGEAIVLTVPGSERSYDLTGLKPGTEYAVTIYGVKGGRYSPPLSAIFTT

SEQ ID NO: 195 - protein, 89 aa, Artificial Sequence
  CD137 Binding Centyrin
LPAPKNLVVSRVTEDSARLSWTAPDAAFDSFAIFYHEFANPGEAIDLPVPGSERSYDLTGLKPGTEYDVRIYGVKGGTASIPLDAEFTT

SEQ ID NO: 196 - protein, 90 aa, Artificial Sequence
  CD137 Binding Centyrin
LPAPKNLVVSRVTEDSARLSWTAPDAAFDSFAIGYVEWTANGEAIVLIVPGSERSYDLTGLKPGTEYVVRIRGGVKGGDSSFPLRADFTT

SEQ ID NO: 197 - protein, 89 aa, Artificial Sequence
  CD137 Binding Centyrin
LPAPKNLVVSRVTEDSARLSWTAPDAAFDSFAISYTESIRQGEAIWLWVPGSERSYDLTGLKPGTEYEVTIGGVKGGIRSYPLWAWFTT

SEQ ID NO: 198 - protein, 89 aa, Artificial Sequence; identical to SEQ ID NO: 78
  CD137 Binding Centyrin

SEQ ID NO: 199 - protein, 89 aa, Artificial Sequence
  CD137 Binding Centyrin
LPAPKNLVVSRVTEDSARLSWTAPDAAFDSFDIPYVEYYPSGEAIVLNVPGSERSYDLTGLKPGTEYGVTIWGIKGGNESVPLTARFTT

SEQ ID NO: 200 - protein, 89 aa, Artificial Sequence
  CD137 Binding Centyrin
LPAPKNLVVSRVTEDSARLSWTAPDAAFDSFAIFYHEFANSGEAIDLPVPGSERSYDLTGLKPGTEYDVRIYGVKGGTASIPLDAEFTT

SEQ ID NO: 201 - protein, 89 aa, Artificial Sequence; identical to SEQ ID NO: 81
  CD137 Binding Centyrin

SEQ ID NO: 202 - protein, 89 aa, Artificial Sequence
  CD137 Binding Centyrin
LPAPKNLVVSRVTEDSARLSWTAPDAAFDSFDIYYLEPWGGGEAIVLTVPGSERSYDLTGLKPGTEYWVTIYGVKVCLGSNPLSAIFTT

SEQ ID NO: 203 - protein, 88 aa, Artificial Sequence
  CD137 Binding Centyrin
LPAPKNLVVSRVTEDSARLSWTAPDAAFDSFEIYYLEGGRGEAIVLTVPGSERSYDLTGLKPGTEYLVTIYGVKCGWASNPLSAIFTT

SEQ ID NO: 204 - protein, 89 aa, Artificial Sequence
  CD137 Binding Centyrin
LPAPKNLVVSRVTEDSARLSWTAPDAAFDSFDIYYYELRLGGEAIVLTVPGSERSYDLTGLKPGTEYLVTIYGVKGCGYSAPLSAIVTT

SEQ ID NO: 205 - protein, 89 aa, Artificial Sequence
  CD137 Binding Centyrin
LPAPKNLVVSRVTEDSARLSWTAPDAAFDSFDIYYYELRLGGEAIVLTVPGSERSYDLTGLKPGTEYLVSIYGVKGCGYSDPLSAIFTT

SEQ ID NO: 206 - protein, 89 aa, Artificial Sequence
  CD137 Binding Centyrin
LPAPKNLVVSRVTEDSARLSWTAPDAAFDSFDIYYYELRLGGEAIVLTVPGSERSYDLTGLKPGTEYLVTIYGVKVCNASTPLSAIFTT

SEQ ID NO: 207 - protein, 89 aa, Artificial Sequence
  CD137 Binding Centyrin
LPAPKNLVVSRVTEDSARLSWTAPDAAFDSFEIYYFELRLGGEAIVLTVPGSERSYDLTGLKPGTEYLVTIYGVKGCGYSDPLSAIFTT

SEQ ID NO: 208 - protein, 89 aa, Artificial Sequence
  CD137 Binding Centyrin
LPAPKNLVVSRVTEDSARLSWTAPDAAFDSFEIYYFELRLGGEAIVLTVPGSERSYDLTGLKPGTEYLVSIYGVKGCGYSDPLSAIFTT

SEQ ID NO: 209 - protein, 89 aa, Artificial Sequence
  CD137 Binding Centyrin
LPAPKNLVVSRVTEDSARLSWTAPDAAFDSFEIYYLELDSDGEAIVLTVPGSERSYDLTGLKPGTEYIVTIYGVKVCTGSRPLSAIFTT

SEQ ID NO: 210 - protein, 89 aa, Artificial Sequence
  CD137 Binding Centyrin
LPAPKNLVVSRVTEDSARLSWTAPDAAFDSFEIYYFELRLGGEAIVLTVPGSERSYDLTGLKPGTEYLVTIYGVKGGGYSTPLSAIFTT

SEQ ID NO: 211 - protein, 89 aa, Artificial Sequence
  CD137 Binding Centyrin
LPAPKNLVVSRVTEDSARLSWTAPDAAFDSFDIYYYELRLGGEAIVLTVPGSERSYDLTGLKPGTEYLVTIYGVKVCEQSYPLSAIFTT

SEQ ID NO: 212 - protein, 89 aa, Artificial Sequence
  CD137 Binding Centyrin
LPAPKNLVVSRVTEDSARLSWTAPDAAFDSFDIYYLESGRDGEAIVLTVPGSERSYDLTGLKPGTEYLVSIYGVKGCGYSDPLSAIFTT

SEQ ID NO: 213 - protein, 89 aa, Artificial Sequence
  CD137 Binding Centyrin
LPAPKNLVVSRVTEDSARLSWTAPDAAFDSFEIYYLEWCSGGEAIVLTVPGSERSYDLTGLKPGTEYLVTIYGVKGCAASDPLSAIFTT

SEQ ID NO: 214 - protein, 89 aa, Artificial Sequence
  CD137 Binding Centyrin
LPAPKNLVVSRVTEDSARLSWTAPDAAFDSFEIYYFELRLGGEAIVLTVPGSERSYDLTGLKPGTEYLVTIYGVKGGAYSNPLSAIFTT

SEQ ID NO: 215 - protein, 89 aa, Artificial Sequence
  CD137 Binding Centyrin
LPAPKNLVVSRVTEDSARLSWTAPDAAFDSFEIYYAEFGYYGEAIVLTVPGSERSYDLTGLKPGTEYLVTIYGVKGCAASDPLSAIFTT

SEQ ID NO: 216 - protein, 89 aa, Artificial Sequence
  CD137 Binding Centyrin
LPAPKNLVVSRVTEDSARLSWTAPDAAFDSFDIYYYELRLGGEAIVLTVPGSERSYDLTGLKPGTEYLVTIYGVKGGDYSPPLSAIFTT

SEQ ID NO: 217 - protein, 89 aa, Artificial Sequence; identical to SEQ ID NO: 98
  CD137 Binding Centyrin

SEQ ID NO: 218 - protein, 89 aa, Artificial Sequence
  CD137 Binding Centyrin
LPAPKNLVVSRVTEDSARLSWTAPDAAFDSFDIYYYELRLGGEAIVLTVPGSERSYDLTGLKPGTEYLVTIYGVKVCYYSTPLSAIFTT

SEQ ID NO: 219 - protein, 89 aa, Artificial Sequence
  CD137 Binding Centyrin
LPAPKNLVVSRVTEDSARLSWTAPDAAFDSFEIYYFELRLGGEAIVLTVPGSERSYDLTGLKPGTEYLVTIYGVKGGDYSPPLSAISTT

SEQ ID NO: 220 - protein, 89 aa, Artificial Sequence
  CD137 Binding Centyrin
LPAPKNLVVSRVTEDSARLSWTAPDAAFDSFEIYYFELRLGGEAIVLTVPGSERSYDLTGLKPGTEYLVTIYGVKGGDYSPPLSAIFTT

SEQ ID NO: 221 - protein, 89 aa, Artificial Sequence
  CD137 Binding Centyrin
LPAPKNLVVSRVTEDSARLSWTAPDAAFDSFDIYYYELRLGGEAIVLTVPGSERSYDLTGLKPGTEYLVTIYGVKGCAASDPLSAIFTT

SEQ ID NO: 222 - protein, 89 aa, Artificial Sequence
  CD137 Binding Centyrin
LPAPKNLVVSRVTEDSARLSWTAPDAAFDSFDIYYYELRLGGEAIVLTVPGSERSYDLTGLKPGTEYLVTIYGVKVCEQSYPLSAISTT

SEQ ID NO: 223 - protein, 89 aa, Artificial Sequence
  CD137 Binding Centyrin
LPAPKNLVVSRVTEDSARLSWTAPDAAFDSFDIYYYELRLGGEAIVLTVPGSERSYDLTGLKPGTEYLVTIYGVKVCLGSNPLSAIFTT

SEQ ID NO: 224 - protein, 89 aa, Artificial Sequence
  CD137 Binding Centyrin
LPAPKNLVVSRVTEDSARLSWTAPDAAFDSFEIYYREPHYGGEAIVLTVPGSERSYDLTGLKPGTEYWVTIYGVKVCLGSNPLSAIFTT